European Patent Application EP 4 458 848 A1, published November 6, 2024. Title: Blood-brain barrier penetrating fusion protein and use thereof. Applicant: IMNEWRUN, Inc. The sequence listing filed with the application follows.

SEQUENCE LISTING (43 sequences)

SEQ ID NO: 1 - protein, 760 aa, Homo sapiens
MMDQARSAFSNLFGGEPLSYTRFSLARQVDGDNSHVEMKLAVDEEENADNNTKANVTKPKRCSGSICYGTIAVIVFFLIGFMIGYLGYCKGVEPKTECERLAGTESPVREEPGEDFPAARRLYWDDLKRKLSEKLDSTDFTGTIKLLNENSYVPREAGSQKDENLALYVENQFREFKLSKVWRDQHFVKIQVKDSAQNSVIIVDKNGRLVYLVENPGGYVAYSKAATVTGKLVHANFGTKKDFEDLYTPVNGSIVIVRAGKITFAEKVANAESLNAIGVLIYMDQTKFPIVNAELSFFGHAHLGTGDPYTPGFPSFNHTQFPPSRSSGLPNIPVQTISRAAAEKLFGNMEGDCPSDWKTDSTCRMVTSESKNVKLTVSNVLKEIKILNIFGVIKGFVEPDHYVVVGAQRDAWGPGAAKSGVGTALLLKLAQMFSDMVLKDGFQPSRSIIFASWSAGDFGSVGATEWLEGYLSSLHLKAFTYINLDKAVLGTSNFKVSASPLLYTLIEKTMQNVKHPVTGQFLYQDSNWASKVEKLTLDNAAFPFLAYSGIPAVSFCFCEDTDYPYLGTTMDTYKELIERIPELNKVARAAAEVAGQFVIKLTHDVELNLDYERYNSQLLSFVRDLNQYRADIKEMGLSLQWLYSARGDFFRATSRLTTDFGNAEKTDRFVMKKLNDRVMRVEYHFLSPYVSPKESPFRHVFWGSGSHTLPALLENLKLRKQNNGAFNETLFRNQLALATWTIQGAANALSGDVWDIDNEF

SEQ ID NO: 2 - protein, 60 aa, Homo sapiens
ELNLDYERYNSQLLSFVRDLNQYRADIKEMGLSLQWLYSARGDFFRATSRLTTDFGNAEK

SEQ ID NO: 3 - protein, 16 aa, synthetic construct
GHHERLKSDEWSVTSG

SEQ ID NO: 4 - protein, 16 aa, synthetic construct
SREERLEEDRRRVDSG

SEQ ID NO: 5 - protein, 16 aa, synthetic construct
TREAARRADEAEVDAG

SEQ ID NO: 6 - protein, 16 aa, synthetic construct
GHDEKLKSDEKLVYSQ

SEQ ID NO: 7 - protein, 16 aa, synthetic construct
SREERRLADEQEVLSG

SEQ ID NO: 8 - protein, 16 aa, synthetic construct
SREAALAADEAAVESG

SEQ ID NO: 9 - protein, 16 aa, synthetic construct
GLDEKLKSDETLVYSQ

SEQ ID NO: 10 - protein, 16 aa, synthetic construct
SEEERRQEDEEEVERG

SEQ ID NO: 11 - protein, 18 aa, synthetic construct
SHLERTKSDEWSIISEGL

SEQ ID NO: 12 - protein, 16 aa, synthetic construct
SREERLREDERRVEEG

SEQ ID NO: 13 - protein, 16 aa, synthetic construct
SREERLREDEEEVESG

SEQ ID NO: 14 - protein, 16 aa, synthetic construct
SREERLEEDKQRVDSG

SEQ ID NO: 15 - protein, 16 aa, synthetic construct
SREERLQQDEQEVDQG

SEQ ID NO: 16 - protein, 16 aa, synthetic construct
SAEEERQRDREEVDNG

SEQ ID NO: 17 - protein, 16 aa, synthetic construct
TAEEERQANEELVEAG

SEQ ID NO: 18 - protein, 16 aa, synthetic construct
GLQEKLKSDEWSVLSQ

SEQ ID NO: 19 - protein, 16 aa, synthetic construct
SREERRREDEREVEEG

SEQ ID NO: 20 - protein, 16 aa, synthetic construct
SREERLREDEEEVDAG

SEQ ID NO: 21 - protein, 16 aa, synthetic construct
GLQEKLKSDEKLVHSQ

SEQ ID NO: 22 - protein, 16 aa, synthetic construct
GDEEKLKSDEELVDSQ

SEQ ID NO: 23 - protein, 16 aa, synthetic construct
SREERRQADEEEVDSG

SEQ ID NO: 24 - protein, 16 aa, synthetic construct
SEEEEREEDEEEVESG

SEQ ID NO: 25 - protein, 16 aa, synthetic construct
GLDEKLKSDEKLVDSQ

SEQ ID NO: 26 - protein, 16 aa, synthetic construct
GLDEKLKSDEDLVYSQ

SEQ ID NO: 27 - protein, 18 aa, synthetic construct
SHHERLKSDEWSVTSGGL

SEQ ID NO: 28 - protein, 16 aa, synthetic construct
SHHERLKSDEWSVTSG

SEQ ID NO: 29 - protein, 18 aa, synthetic construct
SHHERLKSDKWDVESGGL

SEQ ID NO: 30 - protein, 27 aa, synthetic construct
LGHHERLKSDEWSVTSGGLIESESAET

SEQ ID NO: 31 - protein, 36 aa, synthetic construct
ESKAVKWSALGHHERLKSDEWSVTSGGLIESESAET

SEQ ID NO: 32 - protein, 16 aa, synthetic construct
SHHERLKSDEWNVTSR

SEQ ID NO: 33 - protein, 14 aa, synthetic construct
HERLKSDEWSVKSG

SEQ ID NO: 34 - protein, 14 aa, synthetic construct
GHHERLKSDEWSVT

SEQ ID NO: 35 - protein, 16 aa, synthetic construct
SHHERLKSDEWSVTSW

SEQ ID NO: 36 - protein, 16 aa, synthetic construct
SHHERLKADEWSVTSG

SEQ ID NO: 37 - protein, 18 aa, synthetic construct
GHHERLKSDEWSVTSGGL

SEQ ID NO: 38 - protein, 18 aa, synthetic construct
SHHERLKSDTWSVESGGL

SEQ ID NO: 39 - protein, 36 aa, synthetic construct
ESKAVKWSALGHHEALKSDEWSVTSGGLIESESAET

SEQ ID NO: 40 - protein, 16 aa, synthetic construct
GHHERLKSDFWSVTSG

SEQ ID NO: 41 - protein, 12 aa, synthetic construct
GHHERLKSDEWS

SEQ ID NO: 42 - protein, 36 aa, synthetic construct
ESKAVKWSALAHHERLKSDEWSVTSGGLIESESAET

SEQ ID NO: 43 - protein, 16 aa, synthetic construct
GHHERLKSHQWEVESG